European Patent Application EP 4 365 283 A1, published May 8, 2024. Title: C0951ANP0001. Applicant: NATIONAL UNIVERSITY CORPORATION CHIBA UNIVERSITY Kyoto University. The sequence listing filed with the application follows.

SEQUENCE LISTING (5 sequences)

SEQ ID NO: 1 - DNA, 1319 bp, Homo sapiens
atgcccctcaacgttagcttcaccaacaggaactatgacctcgactacgactcggtgcagccgtatttctactgcgacgaggaggagaacttctaccagcagcagcagcagagcgagctgcagcccccggcgcccagcgaggatatctggaagaaattcgagctgctgcccaccccgcccctgtcccctagccgccgctccgggctctgctcgccctcctacgttgcggtcacacccttctcccttcggggagacaacgacggcggtggcgggagcttctccacggccgaccagctggagatggtgaccgagctgctgggaggagacatggtgaaccagagtttcatctgcgacccggacgacgagaccttcatcaaaaacatcatcatccaggactgtatgtggagcggcttctcggccgccgccaagctcgtctcagagaagctggcctcctaccaggctgcgcgcaaagacagcggcagcccgaaccccgcccgcggccacagcgtctgctccacctccagcttgtacctgcaggatctgagcgccgccgctcagagtgcatcgacccctcggtggtcttcccctaccctctcaacgacagcagctcgcccaagtcctgcgcctcgcaagactccagcgccttctctccgtcctcggattctctgctctcctcgacggagtcctccccgcagggcagccccgagcccctggtgctccatgaggagacaccgcccaccaccagcagcgactctgaggaggaacaagaagatgaggaagaaatcgatgttgtttctgtggaaaagaggcaggctcctggcaaaaggtcagagtctggatcaccttctgctggaggccacagcaaacctcctcacagcccactggtcctcaagaggtgccacgtctccacacatcagcacaactacgcagcgcctccctccactcggaaggactatcctgctgccaagagggtcaagttggacagtgtcagagtcctgagacagatcagcaacaaccgaaaatgcaccagccccaggtcctcggacaccgaggagaatgtcaagaggcgaacacacaacgtcttggagcgccagaggaggaacgagctaaaacggagcttttttgccctgcgtgaccagatcccggagttggaaaacaatgaaaaggcccccaaggtagttatccttaaaaaagccacagcatacatcctgtccgtccaagcagaggagcaaaagctcatttctgaagaggacttgttgcggaaacgacgagaacagttgaaacacaaacttgaacagctacggaactcttgtgcgtaa

SEQ ID NO: 2 - DNA, 981 bp, Homo sapiens
atgcatcgaacaacgagaatcaagatcactgagctaaatccccacctgatgtgtgtgctttgtggagggtacttcattgatgccacaaccataatagaatgtctacattccttctgtaaaacgtgtattgttcgttacctggagaccagcaagtattgtcctatttgtgatgtccaagttcacaagaccagaccactactgaatataaggtcagataaaactctccaagatattgtatacaaattagttccagggcttttcaaaaatgaaatgaagagaagaagggatttttatgcagctcatccttctgctgatgctgccaatggctctaatgaagatagaggagaggttgcagatgaagataagagaattataactgatgatgagataataagcttatccattgaattctttgaccagaacagattggatcggaaagtaaacaaagacaaagagaaatctaaggaggaggtgaatgataaaagatacttacgatgcccagcagcaatgactgtgatgcacttaagaaagtttctcagaagtaaaatggacatacctaatactttccagattgatgtcatgtatgaggaggaacctttaaaggattattatacactaatggatattgcctacatttatacctggagaaggaatggtccacttccattgaaatacagagttcgacctacttgtaaaagaatgaagatcagtcaccagagagatggactgacaaatgctggagaactggaaagtgactctgggagtgacaaggccaacagcccagcaggaggtattccctccacctcttcttgtttgcctagccccagtactccagtgcagtctcctcatccacagtttcctcacatttccagtactatgaatggaaccagcaacagccccagcggtaaccaccaatcttcttttgccaatagacctcgaaaatcatcagtaaatgggtcatcagcaacttcttctggttga

SEQ ID NO: 3 - DNA, 702 bp, Homo sapiens
atgtctcagagcaaccgggagctggtggttgactttctctcctacaagctttcccagaaaggatacagctggagtcagtttagtgatgtggaagagaacaggactgaggccccagaagggactgaatcggagatggagacccccagtgccatcaatggcaacccatcctggcacctggcagacagccccgcggtgaatggagccactggccacagcagcagtttggatgcccgggaggtgatccccatggcagcagtaaagcaagcgctgagggaggcaggcgacgagtttgaactgcggtaccggcgggcattcagtgacctgacatcccagctccacatcaccccagggacagcatatcagagctttgaacaggtagtgaatgaactcttccgggatggggtaaactggggtcgcattgtggcctttttctccttcggcggggcactgtgcgtggaaagcgtagacaaggagatgcaggtattggtgagtcggatcgcagcttggatggccacttacctgaatgaccacctagagccttggatccaggagaacggcggctgggatacttttgtggaactctatgggaacaatgcagcagccgagagccgaaagggccaggaacgcttcaaccgctggttcctgacgggcatgactgtggccggcgtggttctgctgggctcactcttcagtcggaaatga

SEQ ID NO: 4 - DNA, 597 bp, Homo sapiens
atgtggggagtattcaggagacagacaactcactcgtcaaatcctccccttcctggccaacaaagctgctgcaaccacagggatttcttctgttcaggcgccatgtcagaaccggctggggatgtccgtcagaacccatgcggcagcaaggcctgccgccgcctcttcggcccagtggacagcgagcagctgagccgcgactgtgatgcgctaatggcgggctgcatccaggaggcccgtgagcgatggaacttcgactttgtcaccgagacaccactggagggtgacttcgcctgggagcgtgtgcggggccttggcctgcccaagctctaccttcccacggggccccggcgaggccgggatgagttgggaggaggcaggcggcctggcacctcacctgctctgctgcaggggacagcagaggaagaccatgtggacctgtcactgtcttgtacccttgtgcctcgctcaggggagcaggctgaagggtccccaggtggacctggagactctcagggtcgaaaacggcggcagaccagcatgacagatttctaccactccaaacgccggctgatcttctccaagaggaagccctaa

SEQ ID NO: 5 - DNA, 1182 bp, Homo sapiens
atggaggagccgcagtcagatcctagcgtcgagccccctctgagtcaggaaacattttcagacctatggaaactacttcctgaaaacaacgttctgtcccccttgccgtcccaagcaatggatgatttgatgctgtccccggacgatattgaacaatggttcactgaagacccaggtccagatgaagctcccagaatgccagaggctgctccccccgtggcccctgcaccagcagctcctacaccggcggcccctgcaccagccccctcctggcccctgtcatcttctgtcccttcccagaaaacctaccagggcagctacggtttccgtctgggcttcttgcattctgggacagccaagtctgtgacttgcacgtactcccctgccctcaacaagatgttttgccaactggccaagacctgccctgtgcagctgtgggttgattccacacccccgcccggcacccgcgtccgcgccatggccatctacaagcagtcacagcacatgacggaggttgtgaggcgctgcccccaccatgagcgctgctcagatagcgatggtctggcccctcctcagcatcttatccgagtggaaggaaatttgcgtgtggagtatttggatgacagaaacacttttcgacatagtgtggtggtgccctatgagccgcctgaggttggctctgactgtaccaccatccactacaactacatgtgtaacagttcctgcatgggcggcatgaaccggaggcccatcctcaccatcatcacactggaagactccagtggtaatctactgggacggaacagctttgaggtgcgtgtttgtgcctgtcctgggagagaccggcgcacagaggaagagaatctccgcaagaaaggggagcctcaccacgagctgcccccagggagcactaagcgagcactgcccaacaacaccagctcctctccccagccaaagaagaaaccactggatggagaatatttcacccttcagatccgtgggcgtgagcgcttcgagatgttccgagagctgaatgaggccttggaactcaaggatgcccaggctgggaaggagccaggggggagcagggctcactccagccacctgaagtccaaaaagggtcagtctacctcccgccataaaaaactcatgttcaagacagaagggcctgactcagactga